European Patent Application EP 4 529 928 A2, published April 2, 2025. Title: COMPOSITIONS, METHODS AND USES OF MESSENGER RNA. Applicant: Translate Bio, Inc. The sequence listing filed with the application follows.

SEQUENCE LISTING (15 sequences)

SEQ ID NO: 1 - RNA, 140 nt, synthetic construct
  source 1..140: mol_type = other RNA
ggacagatcgcctggagacgccatccacgctgttttgacctccatagaagacaccgggaccgatccagcctccgcggccgggaacggtgcattggaacgcggattccccgtgccaagagtgactcaccgtccttgacacg

SEQ ID NO: 2 - RNA, 105 nt, synthetic construct
  source 1..105: mol_type = other RNA
cgggtggcatccctgtgacccctccccagtgcctctcctggccctggaagttgccactccagtgcccaccagccttgtcctaataaaattaagttgcatcaagct

SEQ ID NO: 3 - RNA, 105 nt, synthetic construct
  source 1..105: mol_type = other RNA
gggtggcatccctgtgacccctccccagtgcctctcctggccctggaagttgccactccagtgcccaccagccttgtcctaataaaattaagttgcatcaaagct

SEQ ID NO: 4 - protein, 874 aa, synthetic construct
MQDLHAIQLQLEEEMFNGGIRRFEADQQRQIAAGSESDTAWNRRLLSELIAPMAEGIQAYKEEYEGKKGRAPRALAFLQCVENEVAAYITMKVVMDMLNTDATLQAIAMSVAERIEDQVRFSKLEGHAAKYFEKVKKSLKASRTKSYRHAHNVAVVAEKSVAEKDADFDRWEAWPKETQLQIGTTLLEILEGSVFYNGEPVFMRAMRTYGGKTTYYLQTSESVGQWISAFKEHVAQLSPAYAPCVIPPRPWRTPFNGGFHTEKVASRIRLVKGNREHVRKLTQKQMPKVYKAINALONTQWQINKDVLAVIEEVIRLDLGYGVPSFKPLIDKENKPANPVPVEFQHLRGRELKEMLSPEQWQQFINWKGECARLYTAETKRGSKSAAVVRMVGQARKYSAFESIYFVYAMDSRSRVYVQSSTLSPQSNDLGKALLRFTEGRPVNGVEALKWFCINGANLWGWDKKTFDVRVSNVLDEEFQDMCRDIAADPLTFTQWAKADAPYEFLAWCFEYAQYLDLVDEGRADEFRTHLPVHQDGSCSGIQHYSAMLRDEVGAKAVNLKPSDAPQDIYGAVAQVVIKKNALYMDADDATTFTSGSVTLSGTELRAMASAWDSIGITRSLTKKPVMTLPYGSTRLTCRESVIDYIVDLEEKEAQKAVAEGRTANKVHPFEDDRQDYLTPGAAYNYMTALIWPSISEVVKAPIVAMKMIRQLARFAAKRNEGLMYTLPTGFILEQKIMATEMLRVRTCLMGDIKMSLOVETDIVDEAAMMGAAAPNFVHGHDASHLILTVCELVDKGVTSIAVIHDSFGTHADNTLTLRVALKGQMVAMYIDGNALQKLLEEHEVRWMVDTGIEVPEQGEFDLNEIMDSEYVFA

SEQ ID NO: 5 - DNA, 18 bp, synthetic construct
  source 1..18: mol_type = other DNA
atttaggtgacactatag

SEQ ID NO: 6 - DNA, 23 bp, synthetic construct
  source 1..23: mol_type = other DNA
atttaggggacactatagaagag

SEQ ID NO: 7 - DNA, 22 bp, synthetic construct
  source 1..22: mol_type = other DNA
atttaggggacactatagaagg

SEQ ID NO: 8 - DNA, 23 bp, synthetic construct
  source 1..23: mol_type = other DNA
atttaggggacactatagaaggg

SEQ ID NO: 9 - DNA, 20 bp, synthetic construct
  source 1..20: mol_type = other DNA
atttaggtgacactatagaa

SEQ ID NO: 10 - DNA, 22 bp, synthetic construct
  source 1..22: mol_type = other DNA
atttaggtgacactatagaaga

SEQ ID NO: 11 - DNA, 23 bp, synthetic construct
  source 1..23: mol_type = other DNA
atttaggtgacactatagaagag

SEQ ID NO: 12 - DNA, 22 bp, synthetic construct
  source 1..22: mol_type = other DNA
atttaggtgacactatagaagg

SEQ ID NO: 13 - DNA, 23 bp, synthetic construct
  source 1..23: mol_type = other DNA
atttaggtgacactatagaaggg

SEQ ID NO: 14 - DNA, 23 bp, synthetic construct
  source 1..23: mol_type = other DNA
atttaggtgacactatagaagng

SEQ ID NO: 15 - DNA, 24 bp, synthetic construct
  source 1..24: mol_type = other DNA
catacgatttaggtgacactatag